European Patent Specification EP 3 412 765 B1, published January 18, 2023. Title: Method of producing variant filamentous fungi. Applicant: Kao Corporaiton. The sequence listing filed with the application follows.

SEQUENCE LISTING (152 sequences)

SEQ ID NO: 1 - DNA, 1735 bp, Rhizopus delemar
  pdc1
atgcctgctattaaaatcggtcaacatctccttaaccgtcttaaggaaatcaacattgatgttgtctttggtgttcctggtgatttcaacatggtaagcagacaattgaattgaacgagagcctataaacttattatttctatagcccttgttggatatcattgaagatgacccagaacttacctggggtaacaatgccaacgaattgaatgcatcttatgcagctgatggttatgctcgtattcgtggtgcaggtgctgttgtcactacctttggtgtaggtgagctgtctgctgtcaacggtattgctggttcatactctgagatgcttcccgtgattcacatcgtcggtactccttctactaaatcccaagctgccggtgccatgcttcaccactctttgggtgacggtaactttgatgtgttcttcaacatgtcctccatgattgcctgtgcctctgctcacctcaagaaacaaacggccattgcagaaattgaccgtgtgatctcccaagctgttctctccaagcgtacaggttacattggtatccctatcgatctgatcaagactgaggttgaagtacctgagcccattcctgccctcaagaccgaattacccaaaaacccagctgatgtccaagcgattgccttgagagtggtcacggatgcgatcgccaaagcccaattccctgtgattgttgtcgatggctgtgtgcttcgccagagatgccaaaaggcagtacaagcctttatcgaacgtactggtttccctacttatgttgctcctatgggtaagggtgccgttgacgaatcctctgtgagttaccgtggctgctactcgggtaatgtcacattggaagcagtgaatgaagagatcaagcaagccgatttgatcatcgaagtgggctccatcaagtctgatttcaacacgggtaacttttcatactctctcgaccgttccaagacgatcaccttgcactcctttgccaccatcgtgttttgtgctgaataccaaaaggtctccatgctcgaattcattcctctcttgacccaagcccttcccgaacaaccccgtcaattcaacctgggtccccgcccaagacccgtacctatccaacccggtaccgaaatcacccacaactacttttggcacaaggtacccgaattcatggatgagaacgccattgtctgtgccgagaccggtacagctgaatttgcttcactcaacatggacggacccaagggaacgacttatatcacccaattcctctggggctctatcggtttctcagtaggtgccgctgtgggtgctgcgatcgccgctcgtgatcgtcgtgtgtatctctttgtcggtgatggttccttccaattgacctgtcaagaaatctctggcttccttcgccatggtttgacacctgtgatcttcttgctgaacaatgacggttacttgatcgaaaaactcattcacggtcccgaacgtgcctataataactttcaaatgtgggaatacagcaagacgcttgattatttcggtgctcatcttgaacacaacaagtccatgggtgttcctcccgttggcttcgaaggcaaggtagccacacgcgatgaatttgaatccgccatgagacaggttcaagccaatcctgacaagattcatttccttgaagtcattatgcctcaatttgactctcctcgtgaacttgaactcttggttgccaactctgaaaaccgttaa

SEQ ID NO: 2 - DNA, 3006 bp, Artificial Sequence
  LeftTALEN-pdc1
atggactacaaagaccatgacggtgattataaagatcatgacatcgattacaaggatgacgatgacaagatggcccccaagaagaagaggaaggtgggcattcaccgcggggtacctatggtggacttgaggacactcggttattcgcaacagcaacaggagaaaatcaagcctaaggtcaggagcaccgtcgcgcaacaccacgaggcgcttgtggggcatggcttcactcatgcgcatattgtcgcgctttcacagcaccctgcggcgcttgggacggtggctgtcaaataccaagatatgattgcggccctgcccgaagccacgcacgaggcaattgtaggggtcggtaaacagtggtcgggagcgcgagcacttgaggcgctgctgactgtggcgggtgagcttagggggcctccgctccagctcgacaccgggcagctgctgaagatcgcgaagagagggggagtaacagcggtagaggcagtgcacgcctggcgcaatgcgctcaccggggcccccttgaacttgaccccagaccaggtagtcgcaatcgcgaacaataatgggggaaagcaagccctggaaaccgtgcaaaggttgttgccggtcctttgtcaagaccacggcctgactcccgatcaagttgtagcgattgcgtcgcatgacggagggaaacaagcattggagactgtccaacggctccttcccgtgttgtgtcaagcccacggtttgacgcctgcacaagtggtcgccatcgccagccatgatggcggtaagcaggcgctggaaacagtacagcgcctgctgcctgtactgtgccaggatcatggactgaccccagaccaggtagtcgcaatcgcgtcaaacggagggggaaagcaagccctggaaaccgtgcaaaggttgttgccggtcctttgtcaagaccacggcctgaccccagaccaggtagtcgcaatcgcgaacaataatgggggaaagcaagccctggaaaccgtgcaaaggttgttgccggtcctttgtcaagaccatggcctgactcccgatcaagttgtagcgattgcgtcgcatgacggagggaaacaagcattggagactgtccaacggctccttcccgtgttgtgtcaagcccacggtttgacgcctgcacaagtggtcgccatcgccagcaatggcggcggtaagcaggcgctggaaacagtacagcgcctgctgcctgtactgtgccaggatcatggactgaccccagaccaggtagtcgcaatcgcgtcgaacattgggggaaagcaagccctggaaaccgtgcaaaggttgttgccggtcctttgtcaagaccacggcctgaccccagaccaggtagtcgcaatcgcgtcaaacggagggggaaagcaagccctggaaaccgtgcaaaggttgttgccggtcctttgtcaagaccacggcctgactcccgatcaagttgtagcgattgcgtccaacggtggagggaaacaagcattggagactgtccaacggctccttcccgtgttgtgtcaagcccatggattgaccccagaccaggtagtcgcaatcgcgtcaaacattgggggaaagcaagccctggaaaccgtgcaaaggttgttgccggtcctttgtcaagaccacggcctgactcccgatcaagttgtagcgattgcgtcgaacattggagggaaacaagcattggagactgtccaacggctccttcccgtgttgtgtcaagcccacggtttgacgcctgcacaagtggtcgccatcgccagcaatattggcggtaagcaggcgctggaaacagtacagcgcctgctgcctgtactgtgccaggatcatggactgaccccagaccaggtagtcgcaatcgcgtcaaacattgggggaaagcaagccctggaaaccgtgcaaaggttgttgccggtcctttgtcaagaccacggcctgaccccagaccaggtagtcgcaatcgcgtcaaacggagggggaaagcaagccctggaaaccgtgcaaaggttgttgccggtcctttgtcaagaccacggcctgactcccgatcaagttgtagcgattgcgtcgcatgacggagggaaacaagcattggagactgtccaacggctccttcccgtgttgtgtcaagcccacggtctgacacccgaacaggtggtcgccattgctaataataacggaggacggccagccttggagtccatcgtagcccaattgtccaggcccgatcccgcgttggctgcgttaacgaatgaccatctggtggcgttggcatgtcttggtggacgacccgcgctcgatgcagtcaaaaagggtctgcctcatgctcccgcattgatcaaaagaaccaaccggcggattcccgagagaacttcccatcgagtcgcgggatcccaactagtcaaaagtgaactggaggagaagaaatctgaacttcgtcataaattgaaatatgtgcctcatgaatatattgaattaattgaaattgccagaaattccactcaggatagaattcttgaaatgaaggtaatggaattttttatgaaagtttatggatatagaggtaaacatttgggtggatcaaggaaaccggacggagcaatttatactgtcggatctcctattgattacggtgtgatcgtggatactaaagcttatagcggaggttataatctgccaattggccaagcagatgaaatgcaacgatatgtcgaagaaaatcaaacacgaaacaaacatatcaaccctaatgaatggtggaaagtctatccatcttctgtaacggaatttaagtttttatttgtgagtggtcactttaaaggaaactacaaagctcagcttacacgattaaatcatatcactaattgtaatggagctgttcttagtgtagaagagcttttaattggtggagaaatgattaaagccggcacattaaccttagaggaagtcagacggaaatttaataacggcgagataaacttttaa

SEQ ID NO: 3 - DNA, 3006 bp, Artificial Sequence
  RightTALEN-pdc1
atggactacaaagaccatgacggtgattataaagatcatgacatcgattacaaggatgacgatgacaagatggcccccaagaagaagaggaaggtgggcattcaccgcggggtacctatggtggacttgaggacactcggttattcgcaacagcaacaggagaaaatcaagcctaaggtcaggagcaccgtcgcgcaacaccacgaggcgcttgtggggcatggcttcactcatgcgcatattgtcgcgctttcacagcaccctgcggcgcttgggacggtggctgtcaaataccaagatatgattgcggccctgcccgaagccacgcacgaggcaattgtaggggtcggtaaacagtggtcgggagcgcgagcacttgaggcgctgctgactgtggcgggtgagcttagggggcctccgctccagctcgacaccgggcagctgctgaagatcgcgaagagagggggagtaacagcggtagaggcagtgcacgcctggcgcaatgcgctcaccggggcccccttgaacttgaccccagaccaggtagtcgcaatcgcgtcaaacggagggggaaagcaagccctggaaaccgtgcaaaggttgttgccggtcctttgtcaagaccacggcctgactcccgatcaagttgtagcgattgcgaataacaatggagggaaacaagcattggagactgtccaacggctccttcccgtgttgtgtcaagcccacggtttgacgcctgcacaagtggtcgccatcgccagcaatattggcggtaagcaggcgctggaaacagtacagcgcctgctgcctgtactgtgccaggatcatggactgaccccagaccaggtagtcgcaatcgcgtcaaacggagggggaaagcaagccctggaaaccgtgcaaaggttgttgccggtcctttgtcaagaccacggcctgaccccagaccaggtagtcgcaatcgcgtcaaacggagggggaaagcaagccctggaaaccgtgcaaaggttgttgccggtcctttgtcaagaccacggcctgactcccgatcaagttgtagcgattgcgtcgaacggtggagggaaacaagcattggagactgtccaacggctccttcccgtgttgtgtcaagcccacggtttgacgcctgcacaagtggtcgccatcgccagccatgatggcggtaagcaggcgctggaaacagtacagcgcctgctgcctgtactgtgccaggatcatggactgaccccagaccaggtagtcgcaatcgcgtcacatgacgggggaaagcaagccctggaaaccgtgcaaaggttgttgccggtcctttgtcaagaccacggcctgaccccagaccaggtagtcgcaatcgcgtcaaacggagggggaaagcaagccctggaaaccgtgcaaaggttgttgccggtcctttgtcaagaccacggcctgactcccgatcaagttgtagcgattgcgtccaacggtggagggaaacaagcattggagactgtccaacggctccttcccgtgttgtgtcaagcccatggattgaccccagaccaggtagtcgcaatcgcgtcaaacattgggggaaagcaagccctggaaaccgtgcaaaggttgttgccggtcctttgtcaagaccacggcctgactcccgatcaagttgtagcgattgcgtcgaacattggagggaaacaagcattggagactgtccaacggctccttcccgtgttgtgtcaagcccacggtttgacgcctgcacaagtggtcgccatcgccaacaacaacggcggtaagcaggcgctggaaacagtacagcgcctgctgcctgtactgtgccaggatcatggactgaccccagaccaggtagtcgcaatcgcgtcaaacattgggggaaagcaagccctggaaaccgtgcaaaggttgttgccggtcctttgtcaagaccacggcctgaccccagaccaggtagtcgcaatcgcgtcacatgacgggggaaagcaagccctggaaaccgtgcaaaggttgttgccggtcctttgtcaagaccatggcctgactcccgatcaagttgtagcgattgcgaataacaatggagggaaacaagcattggagactgtccaacggctccttcccgtgttgtgtcaagcccacggtctgacacccgaacaggtggtcgccattgctaataataacggaggacggccagccttggagtccatcgtagcccaattgtccaggcccgatcccgcgttggctgcgttaacgaatgaccatctggtggcgttggcatgtcttggtggacgacccgcgctcgatgcagtcaaaaagggtctgcctcatgctcccgcattgatcaaaagaaccaaccggcggattcccgagagaacttcccatcgagtcgcgggatcccaactagtcaaaagtgaactggaggagaagaaatctgaacttcgtcataaattgaaatatgtgcctcatgaatatattgaattaattgaaattgccagaaattccactcaggatagaattcttgaaatgaaggtaatggaattttttatgaaagtttatggatatagaggtaaacatttgggtggatcaaggaaaccggacggagcaatttatactgtcggatctcctattgattacggtgtgatcgtggatactaaagcttatagcggaggttataatctgccaattggccaagcagatgaaatgcaacgatatgtcgaagaaaatcaaacacgaaacaaacatatcaaccctaatgaatggtggaaagtctatccatcttctgtaacggaatttaagtttttatttgtgagtggtcactttaaaggaaactacaaagctcagcttacacgattaaatcatatcactaattgtaatggagctgttcttagtgtagaagagcttttaattggtggagaaatgattaaagccggcacattaaccttagaggaagtcagacggaaatttaataacggcgagataaacttttaa

SEQ ID NO: 4 - DNA, 1733 bp, Rhizopus delemar
  pdc2
atgccttctatccaaatcggtcaacatcttcttaaccgtctcaaggaaattaacattgatgtagtctttggtgttcctggtgacttcaacatggtaaatgaatataaagagtgatgaacaagttgtatttatatccttcttagcctttactggatatcattgaagacgacccaaagcttacgtggggtaataatgctaatgaattgaacgcttcttatgcagctgatggttatgctcgtattcgtggtgcgggtgctgtcgtcactacgtttggtgttggtgaactctctgctgtgaatggtgttgctggttcttatgctgagatgcttcctgtgattcacattgtcggcacaccttctactaaatctcaagctgctggtgctatgcttcaccactctctgggtgatggtaattttgatgtgttcttcaacatgtcctccatgattgcctgtgcatctactcatctcaagaagcagactgctatcgcagaaattgaccgtgtcatctctcaagctgtcctctcaaaacgtacgggttacatcggtatccctattgacttgatcaagaccgaagtcgaaattccagaggaattaagtcctcttcagaccacacttcccaagaacaacccagaagtccaagcgatcgccttgaaggtcgtcaccgaagccattcagtctgccaagcatcctgtgatcattgtcgatggctgtgtccttcgtcaccgctgtcagaaacccgtccaggaattcatcacccgttccggtttcccaacctacgtggctcccatgggcaagggcgccgtggatgagtccattgagaatttccgtggttgttattcgggtaacgtgacactggaggctgtcaatgaagaaatcaaactggccgatttgattattgagattggttcgatcaagtctgatttcaacacaggtaacttttcatactccctcgatcgttccaagacgatcaccttgcattcttttgctacgatcgtgttttgtgcagagtaccaaaaggtctccatgatggaattcattcctctcttgacccaggcccttccccaacaacctcgtatgttcaacttgggtccacgtgcaaagcctgtgccgatccaacccggaactgaaatcacccacaattacttttggcacaaggtacccgagtacatggaagaaaacgcgattgtctgtgcagagaccggtacagccgaatttgcttcactcaacatggatggtcccaagggtacgacatatatcacccaaatcctttggggttctatcggtttcacggtaggtgcctctgtaggtgccgctatcgccgctcgtgatcgtcgtgtgtatctctttgtcggtgatggttccttccaactgacctgccaagaaatcgctgttttccttcgtcatggcctcacacctgtcatcttcttgctgaacaatgacggttacttgattgaaaaactcattcacggtcctgatcgtgcttacaataattaccaaatgtggaattaccacaagacccttgactatttcggtgctcatcttgaacacaacaagtccatgggtgttcctcccgttggtttcgaaggcaaggtggccacacgtgatgaattcgaatcggccatgaagcaagttcaagccaaccctaacaagattcatttccttgaagtcattatgcctcaatttgatgcccctcgtgaacttgaattattggttgccaactctgaaaaccgataa

SEQ ID NO: 5 - DNA, 3075 bp, Artificial
  LeftTALEN-pdc2
atgggaaaacctattcctaatcctctgctgggcctggattctaccggaggcatggcccctaagaaaaagcggaaggtggacggcggagtggacctgagaacactgggatattctcagcagcagcaggagaagatcaagcccaaggtgagatctacagtggcccagcaccacgaagccctggtgggacacggatttacacacgcccacattgtggccctgtctcagcaccctgccgccctgggaacagtggccgtgaaatatcaggatatgattgccgccctgcctgaggccacacacgaagccattgtgggagtgggaaaacagtggtctggagccagagccctggaagccctgctgacagtggccggagaactgagaggacctcctctgcagctggatacaggacagctgctgaagattgccaaaaggggcggagtgaccgcggtggaagccgtgcacgcctggagaaatgccctgacaggagcccctctgaacctgacccccgaacaggtggtggccattgccagcaacaacggcggcaagcaggccctggaaaccgtgcagagactgctgcccgtgctgtgccaggcccatggcctgacacctgaacaggtggtggctatcgcctctaacaacggaggaaaacaggctctggaaacagtgcagcggctgctgcctgtgctgtgtcaggctcacggcttgactccagaacaggtggtggctattgcttccaacggcggggggaaacaggccctggaaactgtgcagcgcctgctgccagtgctgtgccaggctcacggactgacccccgaacaggtggtggccattgccagcaacaacggcggcaagcaggccctggaaaccgtgcagagactgctgcccgtgctgtgccaggcccatggcctgacacctgaacaggtggtggctatcgcctctaacggcggaggaaaacaggctctggaaacagtgcagcggctgctgcctgtgctgtgtcaggctcacggcttgactccagaacaggtggtggctattgcttccaacggcggggggaaacaggccctggaaactgtgcagcgcctgctgccagtgctgtgccaggctcacgggctgacccccgaacaggtggtggccattgccagcaacaacggcggcaagcaggccctggaaaccgtgcagagactgctgcccgtgctgtgccaggcccatggcctgacacctgaacaggtggtggctatcgcctctcacgacggaggaaaacaggctctggaaacagtgcagcggctgctgcctgtgctgtgtcaggctcacggcttgactccagaacaggtggtggctattgcttccaacggcggggggaaacaggccctggaaactgtgcagcgcctgctgccagtgctgtgccaggctcacggcctcactcccgaacaggtggtggccattgccagcaacaacggcggcaagcaggccctggaaaccgtgcagagactgctgcccgtgctgtgccaggcccatggcctgacacctgaacaggtggtggctatcgcctctaacaacggaggaaaacaggctctggaaacagtgcagcggctgctgcctgtgctgtgtcaggctcacggcttgactccagaacaggtggtggctattgcttccaacggcggggggaaacaggccctggaaactgtgcagcgcctgctgccagtgctgtgccaggctcacggactgacccccgaacaggtggtggccattgccagcaacggcggcggcaagcaggccctggaaaccgtgcagagactgctgcccgtgctgtgccaggcccatggcctgacacctgaacaggtggtggctatcgcctctcacgacggaggaaaacaagcactcgagacagtgcagcggctgctgcctgtgctgtgtcaggctcacggcttgactccagaacaggtggtggctattgcttccaacggcggggggaaacaggccctggaaactgtgcagcgcctgctgccagtgctgtgccaggctcacgggctgacccccgaacaggtggtggccattgccagcaacggcggcggcaagcaggccctggaaaccgtgcagagactgctgcccgtgctgtgccaggcccatggcctgacacctgaacaggtggtggctatcgcctctaatatcggaggaaaacaggctctggaaacagtgcagcggctgctgcctgtgctgtgtcaggctcacggcttgactccacagcaggtcgtggcaattgctagcaacggcggcggacggcccgccctggagagcattgtggcccagctgtctagacctgatcctgccctggccgccctgacaaatgatcacctggtggccctggcctgtctgggaggcagacctgccctggatgccgtgaaaaaaggactgcctcacgcccctgccctgatcaagagaacaaatagaagaatccccgagcggacctctcacagagtggccggatcccagctggtgaaatctgagctggaggagaagaagtctgagctgagacacaagctgaagtacgtgcctcacgagtacatcgagctgatcgagatcgccagaaatagcacccaggatagaatcctggagatgaaggtgatggagttcttcatgaaggtgtacggctacagaggaaagcacctgggaggaagcagaaaacctgacggagccatttatacagtgggcagccctatcgattatggcgtgatcgtggatacaaaggcctacagcggaggctacaatctgcctattggacaggccgatgagatgcagagatacgtggaggagaaccagaccaggaacaagcacatcaaccctaacgagtggtggaaggtgtacccttctagcgtgaccgagttcaagttcctgtttgtgagcggccacttcaagggcaattataaggcccagctgaccaggctgaaccacatcacaaattgtaatggcgccgtgctgtctgtggaggaactgctgattggaggagagatgattaaggccggaacactgacactggaggaggtgagaagaaagttcaacaacggcgagatcaacttctga

SEQ ID NO: 6 - DNA, 3075 bp, Artificial
  RightTALEN-pdc2
atgggaaaacctattcctaatcctctgctgggcctggattctaccggaggcatggcccctaagaaaaagcggaaggtggacggcggagtggacctgagaacactgggatattctcagcagcagcaggagaagatcaagcccaaggtgagatctacagtggcccagcaccacgaagccctggtgggacacggatttacacacgcccacattgtggccctgtctcagcaccctgccgccctgggaacagtggccgtgaaatatcaggatatgattgccgccctgcctgaggccacacacgaagccattgtgggagtgggaaaacagtggtctggagccagagccctggaagccctgctgacagtggccggagaactgagaggacctcctctgcagctggatacaggacagctgctgaagattgccaaaaggggcggagtgaccgcggtggaagccgtgcacgcctggagaaatgccctgacaggagcccctctgaacctgacccccgaacaggtggtggccattgccagcaacaacggcggcaagcaggccctggaaaccgtgcagagactgctgcccgtgctgtgccaggcccatggcctgacacctgaacaggtggtggctatcgcctctcacgacggaggaaaacaggctctggaaacagtgcagcggctgctgcctgtgctgtgtcaggctcacggcttgactccagaacaggtggtggctattgcttcccacgacggggggaaacaggccctggaaactgtgcagcgcctgctgccagtgctgtgccaggctcacggactgacccccgaacaggtggtggccattgccagcaacaacggcggcaagcaggccctggaaaccgtgcagagactgctgcccgtgctgtgccaggcccatggcctgacacctgaacaggtggtggctatcgcctctaatatcggaggaaaacaggctctggaaacagtgcagcggctgctgcctgtgctgtgtcaggctcacggcttgactccagaacaggtggtggctattgcttcccacgacggggggaaacaggccctggaaactgtgcagcgcctgctgccagtgctgtgccaggctcacgggctgacccccgaacaggtggtggccattgccagcaacatcggcggcaagcaggccctggaaaccgtgcagagactgctgcccgtgctgtgccaggcccatggcctgacacctgaacaggtggtggctatcgcctctaatatcggaggaaaacaggctctggaaacagtgcagcggctgctgcctgtgctgtgtcaggctcacggcttgactccagaacaggtggtggctattgcttccaacggcggggggaaacaggccctggaaactgtgcagcgcctgctgccagtgctgtgccaggctcacggcctcactcccgaacaggtggtggccattgccagcaacaacggcggcaagcaggccctggaaaccgtgcagagactgctgcccgtgctgtgccaggcccatggcctgacacctgaacaggtggtggctatcgcctctaacggcggaggaaaacaggctctggaaacagtgcagcggctgctgcctgtgctgtgtcaggctcacggcttgactccagaacaggtggtggctattgcttccaacaacggggggaaacaggccctggaaactgtgcagcgcctgctgccagtgctgtgccaggctcacggactgacccccgaacaggtggtggccattgccagcaacatcggcggcaagcaggccctggaaaccgtgcagagactgctgcccgtgctgtgccaggcccatggcctgacacctgaacaggtggtggctatcgcctctaatatcggaggaaaacaagcactcgagacagtgcagcggctgctgcctgtgctgtgtcaggctcacggcttgactccagaacaggtggtggctattgcttccaacggcggggggaaacaggccctggaaactgtgcagcgcctgctgccagtgctgtgccaggctcacgggctgacccccgaacaggtggtggccattgccagccacgacggcggcaagcaggccctggaaaccgtgcagagactgctgcccgtgctgtgccaggcccatggcctgacacctgaacaggtggtggctatcgcctctaatatcggaggaaaacaggctctggaaacagtgcagcggctgctgcctgtgctgtgtcaggctcacggcttgactccacagcaggtcgtggcaattgctagccacgacggcggacggcccgccctggagagcattgtggcccagctgtctagacctgatcctgccctggccgccctgacaaatgatcacctggtggccctggcctgtctgggaggcagacctgccctggatgccgtgaaaaaaggactgcctcacgcccctgccctgatcaagagaacaaatagaagaatccccgagcggacctctcacagagtggccggatcccagctggtgaaatctgagctggaggagaagaagtctgagctgagacacaagctgaagtacgtgcctcacgagtacatcgagctgatcgagatcgccagaaatagcacccaggatagaatcctggagatgaaggtgatggagttcttcatgaaggtgtacggctacagaggaaagcacctgggaggaagcagaaaacctgacggagccatttatacagtgggcagccctatcgattatggcgtgatcgtggatacaaaggcctacagcggaggctacaatctgcctattggacaggccgatgagatgcagagatacgtggaggagaaccagaccaggaacaagcacatcaaccctaacgagtggtggaaggtgtacccttctagcgtgaccgagttcaagttcctgtttgtgagcggccacttcaagggcaattataaggcccagctgaccaggctgaaccacatcacaaattgtaatggcgccgtgctgtctgtggaggaactgctgattggaggagagatgattaaggccggaacactgacactggaggaggtgagaagaaagttcaacaacggcgagatcaacttctga

SEQ ID NO: 7 - DNA, 2298 bp, Rhizopus delemar
  trpC
atgaccactttacttattgacaactacgacagttttacttataatgtctatcaatacttgagctgccaaggcgccaatgtagttgtctacagaaacgacaaaatcaccatttccgaaattgagcaattggctcctcgcaatattgtcatctcacctggccctggccacccttccaccgatgccggtgtctctcgagaggccattcgagcttttgcaggaaagattcccatcttgggtatttgtatgggtcagcaatgtatgtatgaagtgtacggtggtaaagtgtcatatgcaggtgatattgtgcatggcaaggcatccagcatcaagcatgacagtcgaggtatcttcaagggcgttcctcaaaacaacatggtcactcgttaccattcccttgctggcatgccttctactttacctgaaacattagaagtcactgcgactaccgacgatggtatcatcatgggcattcgacacaaggaatacactgtcgaaggtgttcagttccatcctgaaagtatcctttgtgaacacggacatacgatgatcaacaacttcttaagcttgcgtggtggcacctgggaagagaatcctgcagccggtgttgtctttaagaaagctcgttccgaaacacccaaaatcagtgctagtgaatcccaactcgatctctctcagcaacaacctgccgcagcaccttccatcttgacccgcatttactctcaacgactcaaggatgttcaggcagccaaggagattcccggccagacatttgaagatttagaaaaacttttaaagttgcacgtcgccccacctcttcaagacgtcgtcgctcgcgtgcgtcaaagcaagcccgccttgatggccgaagtcaagcgtgcctctccctcgaaaggaaacattgatgtttcggccaacgcggctgagcaggcacttcaatatgctttagcaggtgcaagcgtcgtctctgttctgactgaacccaaatggttccgcggtacgattcatgatatgcatcaggtccgagaggccttgagccatctgcccaaccgtccttgtgtgttgagaaaggattttattgtcgatcgctatcaaatcttggaaggtcgtctgtacggtgctgatactatcttgttgatcgtggccatgctgaatgatgaacaactgcacgaattgtatcactatgcgaaatcattaggtatggaacccttggtcgaagtcaataatacggaagagatggcccgtgccaatgctttgggcgcacgtctggtgggtgttaataatcgcaacttgcacagctttgatgttgatatggaaaccacgagtcgattggtagagatggtgcctgaaggaacgatcttgtgtgcactttctggtattactggacgagctgatgttgaaatgtacgtcaaacagggtgtgcacgctgtcttggtgggtgaagccctgatgcgtgcttggaatttgaaggagtttgtgtctgatttgttgggtcatgaaaagaaggatcctgtgcctgtgtccaaggaatcaaaatcttcactagtcaaggtatgtggtatctctagtgtggatgcagcagttgaagcagccaagtcaggggctgacttgattggtcttatctttgctgaaaagtccaaacgaaaagtgtctttggaaagagctcaagaaatcgtgtcctcagtgcgtgcgttggatattcaagtcaaacgaacgttatcaaatgatgattctcaactggattggttccagatgcacaagcgtctcttggaaaagcgagcaagaaaacctttggtagttggcgtgtttgtgaatcaatcgattgaatacatgactgaggtggcaacgacagtcggactggaccttattcagctgcatggaaccgaatcaacggagcttgcacgctatttacccgtgcctgtcatcaaagctttccatatcgacagtggtgagttcaatgaagctcagataccaaacctaaatcaaccaggctcttatcattatgtcttactggacgctaaagtgcccagcttaccatcggatcaacaaggtggacgtggtgtcaagtttgattggtcaattgctaccaaaatcgtgaaacataggcactttgagtttttgggtaatcaagatttccctgtcatcttggctggtgggttggatcctaccaatgtggcatctgccattcaacaggtgaaaccctggattgtggatgtgtcgagtggtgttgaaacagatggagtgaaggatttagaaaagattcgtgcctttgttaaaactgtccagtcaacacaattttaa

SEQ ID NO: 8 - DNA, 3075 bp, Artificial
  LeftTALEN-trpC
atgggaaaacctattcctaatcctctgctgggcctggattctaccggaggcatggcccctaagaaaaagcggaaggtggacggcggagtggacctgagaacactgggatattctcagcagcagcaggagaagatcaagcccaaggtgagatctacagtggcccagcaccacgaagccctggtgggacacggatttacacacgcccacattgtggccctgtctcagcaccctgccgccctgggaacagtggccgtgaaatatcaggatatgattgccgccctgcctgaggccacacacgaagccattgtgggagtgggaaaacagtggtctggagccagagccctggaagccctgctgacagtggccggagaactgagaggacctcctctgcagctggatacaggacagctgctgaagattgccaaaaggggcggagtgaccgcggtggaagccgtgcacgcctggagaaatgccctgacaggagcccctctgaacctgacccccgaacaggtggtggccattgccagcaacaacggcggcaagcaggccctggaaaccgtgcagagactgctgcccgtgctgtgccaggcccatggcctgacacctgaacaggtggtggctatcgcctctcacgacggaggaaaacaggctctggaaacagtgcagcggctgctgcctgtgctgtgtcaggctcacggcttgactccagaacaggtggtggctattgcttcccacgacggggggaaacaggccctggaaactgtgcagcgcctgctgccagtgctgtgccaggctcacggactgacccccgaacaggtggtggccattgccagcaacatcggcggcaagcaggccctggaaaccgtgcagagactgctgcccgtgctgtgccaggcccatggcctgacacctgaacaggtggtggctatcgcctctaatatcggaggaaaacaggctctggaaacagtgcagcggctgctgcctgtgctgtgtcaggctcacggcttgactccagaacaggtggtggctattgcttccaacaacggggggaaacaggccctggaaactgtgcagcgcctgctgccagtgctgtgccaggctcacgggctgacccccgaacaggtggtggccattgccagcaacaacggcggcaagcaggccctggaaaccgtgcagagactgctgcccgtgctgtgccaggcccatggcctgacacctgaacaggtggtggctatcgcctctcacgacggaggaaaacaggctctggaaacagtgcagcggctgctgcctgtgctgtgtcaggctcacggcttgactccagaacaggtggtggctattgcttccaacaacggggggaaacaggccctggaaactgtgcagcgcctgctgccagtgctgtgccaggctcacggcctcactcccgaacaggtggtggccattgccagccacgacggcggcaagcaggccctggaaaccgtgcagagactgctgcccgtgctgtgccaggcccatggcctgacacctgaacaggtggtggctatcgcctctcacgacggaggaaaacaggctctggaaacagtgcagcggctgctgcctgtgctgtgtcaggctcacggcttgactccagaacaggtggtggctattgcttccaatattggggggaaacaggccctggaaactgtgcagcgcctgctgccagtgctgtgccaggctcacggactgacccccgaacaggtggtggccattgccagcaacatcggcggcaagcaggccctggaaaccgtgcagagactgctgcccgtgctgtgccaggcccatggcctgacacctgaacaggtggtggctatcgcctctaacggcggaggaaaacaagcactcgagacagtgcagcggctgctgcctgtgctgtgtcaggctcacggcttgactccagaacaggtggtggctattgcttccaacaacggggggaaacaggccctggaaactgtgcagcgcctgctgccagtgctgtgccaggctcacgggctgacccccgaacaggtggtggccattgccagcaacggcggcggcaagcaggccctggaaaccgtgcagagactgctgcccgtgctgtgccaggcccatggcctgacacctgaacaggtggtggctatcgcctctaatatcggaggaaaacaggctctggaaacagtgcagcggctgctgcctgtgctgtgtcaggctcacggcttgactccacagcaggtcgtggcaattgctagcaacaacggcggacggcccgccctggagagcattgtggcccagctgtctagacctgatcctgccctggccgccctgacaaatgatcacctggtggccctggcctgtctgggaggcagacctgccctggatgccgtgaaaaaaggactgcctcacgcccctgccctgatcaagagaacaaatagaagaatccccgagcggacctctcacagagtggccggatcccagctggtgaaatctgagctggaggagaagaagtctgagctgagacacaagctgaagtacgtgcctcacgagtacatcgagctgatcgagatcgccagaaatagcacccaggatagaatcctggagatgaaggtgatggagttcttcatgaaggtgtacggctacagaggaaagcacctgggaggaagcagaaaacctgacggagccatttatacagtgggcagccctatcgattatggcgtgatcgtggatacaaaggcctacagcggaggctacaatctgcctattggacaggccgatgagatgcagagatacgtggaggagaaccagaccaggaacaagcacatcaaccctaacgagtggtggaaggtgtacccttctagcgtgaccgagttcaagttcctgtttgtgagcggccacttcaagggcaattataaggcccagctgaccaggctgaaccacatcacaaattgtaatggcgccgtgctgtctgtggaggaactgctgattggaggagagatgattaaggccggaacactgacactggaggaggtgagaagaaagttcaacaacggcgagatcaacttctga

SEQ ID NO: 9 - DNA, 3075 bp, Artificial
  RightTALEN-trpC
atgggaaaacctattcctaatcctctgctgggcctggattctaccggaggcatggcccctaagaaaaagcggaaggtggacggcggagtggacctgagaacactgggatattctcagcagcagcaggagaagatcaagcccaaggtgagatctacagtggcccagcaccacgaagccctggtgggacacggatttacacacgcccacattgtggccctgtctcagcaccctgccgccctgggaacagtggccgtgaaatatcaggatatgattgccgccctgcctgaggccacacacgaagccattgtgggagtgggaaaacagtggtctggagccagagccctggaagccctgctgacagtggccggagaactgagaggacctcctctgcagctggatacaggacagctgctgaagattgccaaaaggggcggagtgaccgcggtggaagccgtgcacgcctggagaaatgccctgacaggagcccctctgaacctgacccccgaacaggtggtggccattgccagccacgacggcggcaagcaggccctggaaaccgtgcagagactgctgcccgtgctgtgccaggcccatggcctgacacctgaacaggtggtggctatcgcctctaacaacggaggaaaacaggctctggaaacagtgcagcggctgctgcctgtgctgtgtcaggctcacggcttgactccagaacaggtggtggctattgcttccaacaacggggggaaacaggccctggaaactgtgcagcgcctgctgccagtgctgtgccaggctcacggactgacccccgaacaggtggtggccattgccagcaacatcggcggcaagcaggccctggaaaccgtgcagagactgctgcccgtgctgtgccaggcccatggcctgacacctgaacaggtggtggctatcgcctctaatatcggaggaaaacaggctctggaaacagtgcagcggctgctgcctgtgctgtgtcaggctcacggcttgactccagaacaggtggtggctattgcttccaatattggggggaaacaggccctggaaactgtgcagcgcctgctgccagtgctgtgccaggctcacgggctgacccccgaacaggtggtggccattgccagcaacggcggcggcaagcaggccctggaaaccgtgcagagactgctgcccgtgctgtgccaggcccatggcctgacacctgaacaggtggtggctatcgcctctaacaacggaggaaaacaggctctggaaacagtgcagcggctgctgcctgtgctgtgtcaggctcacggcttgactccagaacaggtggtggctattgcttccaacaacggggggaaacaggccctggaaactgtgcagcgcctgctgccagtgctgtgccaggctcacggcctcactcccgaacaggtggtggccattgccagcaacggcggcggcaagcaggccctggaaaccgtgcagagactgctgcccgtgctgtgccaggcccatggcctgacacctgaacaggtggtggctatcgcctctaacaacggaggaaaacaggctctggaaacagtgcagcggctgctgcctgtgctgtgtcaggctcacggcttgactccagaacaggtggtggctattgcttccaatattggggggaaacaggccctggaaactgtgcagcgcctgctgccagtgctgtgccaggctcacggactgacccccgaacaggtggtggccattgccagcaacggcggcggcaagcaggccctggaaaccgtgcagagactgctgcccgtgctgtgccaggcccatggcctgacacctgaacaggtggtggctatcgcctctaacggcggaggaaaacaagcactcgagacagtgcagcggctgctgcctgtgctgtgtcaggctcacggcttgactccagaacaggtggtggctattgcttccaacggcggggggaaacaggccctggaaactgtgcagcgcctgctgccagtgctgtgccaggctcacgggctgacccccgaacaggtggtggccattgccagcaacggcggcggcaagcaggccctggaaaccgtgcagagactgctgcccgtgctgtgccaggcccatggcctgacacctgaacaggtggtggctatcgcctctaacaacggaggaaaacaggctctggaaacagtgcagcggctgctgcctgtgctgtgtcaggctcacggcttgactccacagcaggtcgtggcaattgctagcaacggcggcggacggcccgccctggagagcattgtggcccagctgtctagacctgatcctgccctggccgccctgacaaatgatcacctggtggccctggcctgtctgggaggcagacctgccctggatgccgtgaaaaaaggactgcctcacgcccctgccctgatcaagagaacaaatagaagaatccccgagcggacctctcacagagtggccggatcccagctggtgaaatctgagctggaggagaagaagtctgagctgagacacaagctgaagtacgtgcctcacgagtacatcgagctgatcgagatcgccagaaatagcacccaggatagaatcctggagatgaaggtgatggagttcttcatgaaggtgtacggctacagaggaaagcacctgggaggaagcagaaaacctgacggagccatttatacagtgggcagccctatcgattatggcgtgatcgtggatacaaaggcctacagcggaggctacaatctgcctattggacaggccgatgagatgcagagatacgtggaggagaaccagaccaggaacaagcacatcaaccctaacgagtggtggaaggtgtacccttctagcgtgaccgagttcaagttcctgtttgtgagcggccacttcaagggcaattataaggcccagctgaccaggctgaaccacatcacaaattgtaatggcgccgtgctgtctgtggaggaactgctgattggaggagagatgattaaggccggaacactgacactggaggaggtgagaagaaagttcaacaacggcgagatcaacttctga

SEQ ID NO: 10 - DNA, 46 bp, Artificial
  oJK162
cgagctcgaattatttaaatgaacagcaagttaataatctagaggg

SEQ ID NO: 11 - DNA, 39 bp, Artificial Sequence
  oJK163
tatgaccatgattacgatgagaggcaaaatgaagcgtac

SEQ ID NO: 12 - DNA, 30 bp, Artificial
  oJK164
atttaaataattcgagctcggtacccgggg

SEQ ID NO: 13 - DNA, 20 bp, Artificial
  oJK165
cgtaatcatggtcatagctg

SEQ ID NO: 14 - DNA, 29 bp, Artificial
  oJK202
tagagggaaaaagagagaattgaaatagg

SEQ ID NO: 15 - DNA, 31 bp, Artificial Sequence
  oJK204
ttttgttatttaattgtattaattgataatg

SEQ ID NO: 16 - DNA, 36 bp, Artificial Sequence
  oJK205
aattaaataacaaaatcattttaattacgcattttc

SEQ ID NO: 17 - DNA, 37 bp, Artificial
  oJK216
catgattacgcggccgcgccattataatgcactagtg

SEQ ID NO: 18 - DNA, 38 bp, Artificial
  oJK210
ctctttttccctctaatgagaggcaaaatgaagcgtac

SEQ ID NO: 19 - DNA, 31 bp, Artificial
  oJK211
atttaaatgtaatcatggtcatagctgtttc

SEQ ID NO: 20 - DNA, 35 bp, Artificial
  trpC-lost-F
tttaaattagagggaaaaagagagaattgaaatag

SEQ ID NO: 21 - DNA, 35 bp, Artificial
  trpC-lost-R
tccctctaatttaaatgaattcgagctcggtaccc

SEQ ID NO: 22 - DNA, 31 bp, Artificial; identical to SEQ ID NO: 15
  adhpro-R

SEQ ID NO: 23 - DNA, 27 bp, Artificial
  adhter-F
tcattttaattacgcattttcatttac

SEQ ID NO: 24 - DNA, 40 bp, Artificial
  adhpro-TALEN-F
aattaaataacaaaaatggactacaaagaccatgacggtg

SEQ ID NO: 25 - DNA, 40 bp, Artificial
  TAELN-adhter-R
gcgtaattaaaatgattaaaagtttatctcgccgttatta

SEQ ID NO: 26 - DNA, 45 bp, Artificial
  adhpro-LifeTALEN-F
aattaaataacaaaaatgggaaaacctattcctaatcctctgctg

SEQ ID NO: 27 - DNA, 47 bp, Artificial
  LifeTALEN-adhter-R
gcgtaattaaaatgatcagaagttgatctcgccgttgttgaactttc

SEQ ID NO: 28 - DNA, 19 bp, Artificial
  pPTR1-sal1-F
gggtaccgagctcgaattc

SEQ ID NO: 29 - DNA, 20 bp, Artificial
  pPTR1-sal1-R
ggggatcctctagagtcgac

SEQ ID NO: 30 - DNA, 41 bp, Artificial
  sal1-ldhpro-F3
ctctagaggatcccctaggtgtggctgtggtgaccatattg

SEQ ID NO: 31 - DNA, 28 bp, Artificial
  ldhpro-R
gagaattatattgtaaagaaaaataaag

SEQ ID NO: 32 - DNA, 50 bp, Artificial
  ldhpro-exo1-F2
tacaatataattctcatgaaaatccaagttgcttctcctattgaccaatc

SEQ ID NO: 33 - DNA, 51 bp, Artificial
  exo1-pdcter-R2
atgaattctaagattttatcttctttcatgagaaacactaaacttgataac

SEQ ID NO: 34 - DNA, 24 bp, Artificial
  pdcTer-F
aatcttagaattcatctttttttg

SEQ ID NO: 35 - DNA, 39 bp, Artificial
  pdcTer-sal1-R
tcgagctcggtacccactctaccgtctgctcttttgtct

SEQ ID NO: 36 - DNA, 45 bp, Artificial
  adhpro-exo1-F
aattaaataacaaaaatgaaaatccaagttgcttctcctattgac

SEQ ID NO: 37 - DNA, 46 bp, Artificial
  exo1-adhter-R
gcgtaattaaaatgattatcttctttcatgagaaacactaaacttg

SEQ ID NO: 38 - DNA, 34 bp, Artificial
  pUC18-Pae1-F3
ctgcaggtcgactctagaggatccccgggtaccg

SEQ ID NO: 39 - DNA, 35 bp, Artificial
  pUC18-Hind3-R3
gcttggcactggccgtcgttttacaacgtcgtgac

SEQ ID NO: 40 - DNA, 45 bp, Artificial
  PDC1-upstr-F
cggccagtgccaagcgcagacttcaacagttggcttttttaagta

SEQ ID NO: 41 - DNA, 47 bp, Artificial
  PDC1-upstr-R
cattttgcctctcatgtttttaaatttgttttgtagagtattgaata

SEQ ID NO: 42 - DNA, 29 bp, Artificial
  trpCpro-R
gaacagcaagttaataatctagagggcgc

SEQ ID NO: 43 - DNA, 29 bp, Artificial
  trpCter-F
atgagaggcaaaatgaagcgtacaaagag

SEQ ID NO: 44 - DNA, 49 bp, Artificial
  PDC1-downstr-F
attaacttgctgttcaatcttagaattcattttttttttgtatcattcg

SEQ ID NO: 45 - DNA, 49 bp, Artificial
  PDC1-downstr-R
agagtcgacctgcaggcgtcaataagagcttgaaggttggtgccggatc

SEQ ID NO: 46 - DNA, 45 bp, Artificial
  PDC2-upstr-F
cggccagtgccaagcttatgggaaaaatgtgaaaatcatcccact

SEQ ID NO: 47 - DNA, 45 bp, Artificial
  PDC2-upstr-R
cattttgcctctcatgtttagttcaaataatatttttttttgtga

SEQ ID NO: 48 - DNA, 45 bp, Artificial
  PDC2-downstr-F
attaacttgctgttcagttctctttctgtaataatccttgatttc

SEQ ID NO: 49 - DNA, 45 bp, Artificial
  PDC2-downstr-R
agagtcgacctgcagcctttttacagaaaacaagcacatctttac

SEQ ID NO: 50 - DNA, 30 bp, Artificial
  trpC-inactive-F
taacgcatcagttccatcctgaaagtatcc

SEQ ID NO: 51 - DNA, 28 bp, Artificial
  trpC-inactive-R
ggaactgatgcgttaaaaagaggggaaa

SEQ ID NO: 52 - DNA, 29 bp, Artificial
  pdc1ter-F
aatcttagaattcattttttttttgtatc

SEQ ID NO: 53 - DNA, 44 bp, Artificial
  trpC-adh1pro-F
attaacttgctgttctagagggaaaaagagagaattgaaatagg

SEQ ID NO: 54 - DNA, 45 bp, Artificial
  FT1-pdc1Ter-R
atgaattctaagattttaatagaaaccctgcttaaatgcaagacc

SEQ ID NO: 55 - DNA, 45 bp, Artificial
  PYC-pdc1Ter-R
atgaattctaagattttaggcttcctctttgacaaccttggccac

SEQ ID NO: 56 - DNA, 30 bp, Artificial
  PDC1-upstr-F2
gcagacttcaacagttggcttttttaagta

SEQ ID NO: 57 - DNA, 34 bp, Artificial
  PDC1-downstr-R2
gcgtcaataagagcttgaaggttggtgccggatc

SEQ ID NO: 58 - DNA, 20 bp, Artificial
  pdc1-up2
cattcccacaggatttgtgc

SEQ ID NO: 59 - DNA, 25 bp, Artificial
  trpC(d)-1
gtgagatgttgatcatttgtacatg

SEQ ID NO: 60 - DNA, 20 bp, Artificial
  pdc2-down1
agaagacaacctagaccctc

SEQ ID NO: 61 - DNA, 20 bp, Artificial
  trpC(d)-7
atagctcttggtgggattcg

SEQ ID NO: 62 - DNA, 25 bp, Artificial
  pdc1-down3
gctgctcgagatcctccaaggtatc

SEQ ID NO: 63 - DNA, 20 bp, Artificial
  trpC(d)-5
ttcgaccaagggttccatac

SEQ ID NO: 64 - DNA, 34 bp, Artificial; identical to SEQ ID NO: 57
  PDC1-downstr-R-P

SEQ ID NO: 65 - DNA, 30 bp, Artificial
  pdc1_750-F
tagattcaatttgattggataaagttcatc

SEQ ID NO: 66 - DNA, 30 bp, Artificial
  pdc1_750-R-P
ataacaaacaatggctaaaagtggaccccc

SEQ ID NO: 67 - DNA, 30 bp, Artificial
  pdc1_500-F
tttactagtttaaagcaaaaaacatgagca

SEQ ID NO: 68 - DNA, 30 bp, Artificial
  pdc1_500-R-P
ttcaatttacatttctttatgaatatgcct

SEQ ID NO: 69 - DNA, 30 bp, Artificial
  pdc1_250-F
gtgtttatctgttcacaagtactggtaagc

SEQ ID NO: 70 - DNA, 30 bp, Artificial
  pdc1_250-R-P
ttcaatataaaccaagtccctaaaagaaat

SEQ ID NO: 71 - DNA, 30 bp, Artificial
  pdc1_100-F
gctgatatgacattgcgacgaaaatagtat

SEQ ID NO: 72 - DNA, 30 bp, Artificial
  pdc1_100-R-P
aaaaaaaaagcttattttcaaaaatatgat

SEQ ID NO: 73 - DNA, 30 bp, Artificial
  pdc1_50-F
tcgttcaaaaaaaatcattattcaatactc

SEQ ID NO: 74 - DNA, 30 bp, Artificial
  pdc1_50-R-P
gtaatgaagtatagaacgaatgatacaaaa

SEQ ID NO: 75 - DNA, 30 bp, Artificial
  pdc1_45-F
caaaaaaaatcattattcaatactctacaa

SEQ ID NO: 76 - DNA, 32 bp, Artificial
  pdc1_45-R-P
gaagtatagaacgaatgatacaaaaaaaaaat

SEQ ID NO: 77 - DNA, 30 bp, Artificial
  pdc1_40-F
aaaatcattattcaatactctacaaaacaa

SEQ ID NO: 78 - DNA, 30 bp, Artificial
  pdc1_40-R-P
atagaacgaatgatacaaaaaaaaaatgaa

SEQ ID NO: 79 - DNA, 30 bp, Artificial
  pdc1_35-F
cattattcaatactctacaaaacaaattta

SEQ ID NO: 80 - DNA, 30 bp, Artificial
  pdc1_35-R-P
acgaatgatacaaaaaaaaaatgaattcta

SEQ ID NO: 81 - DNA, 30 bp, Artificial
  pdc1_30-F
ttcaatactctacaaaacaaatttaaaaac

SEQ ID NO: 82 - DNA, 30 bp, Artificial
  pdc1_30-R-P
tgatacaaaaaaaaaatgaattctaagatt

SEQ ID NO: 83 - DNA, 30 bp, Artificial
  pdc1_25-F
tactctacaaaacaaatttaaaaacatgag

SEQ ID NO: 84 - DNA, 30 bp, Artificial
  pdc1_25-R-P
caaaaaaaaaatgaattctaagattgaaca

SEQ ID NO: 85 - DNA, 30 bp, Artificial
  pdc1_20-F
tacaaaacaaatttaaaaacatgagaggca

SEQ ID NO: 86 - DNA, 30 bp, Artificial
  pdc1_20-R-P
aaaaaatgaattctaagattgaacagcaag

SEQ ID NO: 87 - DNA, 30 bp, Artificial
  pdc1_15-F
aacaaatttaaaaacatgagaggcaaaatg

SEQ ID NO: 88 - DNA, 30 bp, Artificial
  pdc1_15-R-P
atgaattctaagattgaacagcaagttaat

SEQ ID NO: 89 - DNA, 30 bp, Artificial
  pdc1_10-F
atttaaaaacatgagaggcaaaatgaagcg

SEQ ID NO: 90 - DNA, 30 bp, Artificial
  pdc1_10-R-P
ttctaagattgaacagcaagttaataatct

SEQ ID NO: 91 - DNA, 30 bp, Artificial
  pdc1_5-F
aaaacatgagaggcaaaatgaagcgtacaa

SEQ ID NO: 92 - DNA, 30 bp, Artificial
  pdc1_5-R-P
agattgaacagcaagttaataatctagagg

SEQ ID NO: 93 - DNA, 30 bp, Artificial
  PDC2-upstr-F2
ttatgggaaaaatgtgaaaatcatcccact

SEQ ID NO: 94 - DNA, 30 bp, Artificial
  PDC2-downstr-R2-P
cctttttacagaaaacaagcacatctttac

SEQ ID NO: 95 - DNA, 27 bp, Artificial
  trpC-ki-F2-P
cttttcatgacccaacaaatcagacac

SEQ ID NO: 96 - DNA, 18 bp, Rhizopus delemar
  Target of LeftTALEN-pdc1
tgcctgctattaaaatcg

SEQ ID NO: 97 - DNA, 18 bp, Rhizopus delemar
  Target of RightTALEN-pdc1
ttgatttccttaagacgg

SEQ ID NO: 98 - DNA, 19 bp, Rhizopus delemar
  Target of LeftTALEN-pdc2
tggtgttgctggttcttat

SEQ ID NO: 99 - DNA, 19 bp, Rhizopus delemar
  Target of RightTALEN-pdc2
tgccgacaatgtgaatcac

SEQ ID NO: 100 - DNA, 19 bp, Rhizopus delemar
  Target of LeftTALEN-trpC
tgccaaggcgccaatgtag

SEQ ID NO: 101 - DNA, 19 bp, Rhizopus delemar
  Target of RightTALEN-trpC
tcggaaatggtgattttgt

SEQ ID NO: 102 - DNA, 513 bp, Rhizopus delemar
  FT1
atgtcttctatcgaaacctccaaaatctcaagttttatgatcaacaatattgatgactttgttgcagattggcatgttcgcgttacttggatcgcattcatgacactctgggtcttttggggattggtttgggttttccgcaacttctttgtttcaaactctcctgcattgactcctgctcctgaagcaaatgctgctgatgatacggaagcatcaaagaaaaaactctttagcgttaccagtgacagttttgctcttcgtctagatcgtgctcatcaagttgtaaaagatgccttgttctctcttctctgtcttctttccatgaactcctttgctcgtgcttcaactcgtgctgtcatgatcctcgcttggttcttcactgcctttgctgtctgttggtttgctgtcgtattccttgttgataaccgctttgttcgtttgacgtattcacttgtcttttacgctcttggtcttgctattgccggtcttgcatttaagcagggtttctattaa

SEQ ID NO: 103 - DNA, 3540 bp, Rhizopus delemar
  PYC
atgcctgctgcaccagtacgtgaacactctgtggataccattcgtagaaatagcgaagtgatgggtaacctgagaaaattgatggtggttaatcgtggtgaaattgctatccgtgtctttcgtacagctcatgaactctctatgaagacagtagctattttctctcatgaagatagattatccatgcacagatataaggctgatgaatcctatcaactcggtcgtattggtcaatacacacctgtaggtgcttatctggcacaagatgaagtcgttcgaatcgcaaaggaacgtggtgtgagcatgattcatcctggttatggtttcttgtctgaaaatgctgaattcgctcgcaaggtggaagctgcaggaatcactttcattggtccctctcctgatgtcattgaaagtttaggcgataagacaaaagccagaacgattgccatgaagtgtgaagtccctgttgtccctggcacacctggacccgtcagtgaatacaaagatgccctgaactttatcaaagaatatggttttcctatcatcatcaaggctgccatgggtggtggtggtcgtggtatgcgtgtggttcgtgacgaagccagtctagaggacgcgtttacccgtgcgaaatctgaagctttggctgcctttggtgatggcactgtctttatcgaacgtttccttgataagcctcgtcatatcgaggttcaattgttggcagatcgtgcaggtaacgtggtccatctctttgaacgtgattgctctgttcagcgtcgtcaccaaaaggtcgttgaaatcgcacctgccaaaaacttggataacaaggtacgtgaggccatcttgaacgatgcgatcaagattgccaaggctgtaaagtacaagaatgcgggtactgcagaattcttggtggataaccaaaaccgtcactactttatcgaaatcaatcctcgtatccaagtcgaacataccatcacagaagaaatcacgggtatcgatatcgttgccgctcaaattcagattgctgccggtgccctcttgcctcaattgggtcttacccaacaacgtatccgtcaacgtgggttcgcgatccagtgtcgtgtgacaaccgaggaccccgaaaagaatttccagcctgacacgggtaagatcgaagtttaccgttcctctggtggtaacggtgttcgtctggatggtggtgctggttacgcaggtgctatcattacccctcactatgattcacttttggtcaaagtctcttgttctggatccacctacgaagtcgctcgtcgaaagatcgtccgtgccttggtcgaattcagaatccgtggtgtcaagaccaatatccccttcttacaacgtctcttgacccatgataccttcatcaacggtaactgctggacaactttcattgatgatactcccgatcttttccgtcttgttcaattccaaaaccgtgctcaaagactcttgggttacctgggtgatgtcgtcgtcaatggttctcaaatcaagggtcaaatgggtgatcccattctgaagcaagagatcgaaatccccgtgttgcgtgaaagtggtagtgacaagacggtcgatgtctctgctcctgctacggaaggctggagaaagatcattgtggaacaaggacctgaagctttcgcaaaagctgtccgtgcttaccctggtgtcttgatcaccgataccacctggagagacgctcatcagagtttattggccactcgtgtgagaactgtcgatctcttgcgtatcgcccctgctacctctcacgctttggccaacgccttttcattggaatgttggggaggtgctacgtttgatgttgccatgcgtttccttcatgaagatccttgggaccgtcttgctgctttgcgaaagttggtacccaatgtacccttccaaatgcttttgcgtggtgccaatgcggtaggttacacctcttaccctgataatgttatctatgaattctgtgacaaggcagtcaagtgtggtatggatgtcttccgtatctttgactctctcaattatgttgagaacatgagattgggtattgacgctgtcaagaaggccggtggtgttgttgaagccaccatctgttacacgggtgatgtctccaaccctaaccgcaagaagtacgacttgaagtactaccttgaccttacacaatccttggtgaacgaaggtattcacatcttgggtatcaaggacatggctggtcttctcaaacccgaggcagccaagttactggtctccagtatccgtgccaagttccccgacttgcccatccacgttcacacacacgataccgcaggtacgggtgttgctagcatgatggccgctgccgctgctggtgctgacattgttgatgttgccgtggacgccatgtccggcatgacctctcaaccagcgatgggtgccattgtcgctggactggaacagaccaatttgggtaccggtatccgcatggaagacattcatgccatcaattcttactgggagcaatgccgtttgctttactcttgcttcgaagccaacgtgcgttcggccgattcgggtgtctatgaacatgaaatgcctggtggacaatataccaacttgatgttccaagcccaacaactcggtttgggaactcagtggaagcaaatcaagaaggcttacaaggaggccaacgaactctgtggtgacctggtcaaggtcacgccttcgtccaaggtcgtgggtgatcttgctcaattcatggtttccaaccaactctctgccaaagaatttgaagaacgcgcctcgagtctctctctgcccacctctgtcatcgagttcttccaaggttatctcggtcaaccctatggcggtttccccgagcccttgcgctccaacatccttcgtgatctccctcgcctcgacggtcgccctggtgctagcctgcctccgttggacatggctaaactcaaggaagagttggttgaaaagtacggttcgagcatccgtgattacgacgtgatctcggctgctctttaccccaaggtctttgccgactaccgtgataccgtcagtcaatacggtgatctctccgttttgcctacacgctactttttgtccaagcccgagatcaatgaagaattccatgtggagattgaagaaggaaagacgttgatcatcaagttattggccgtcggtcctctgaacaatgacggtaaacgtgatgtttactttgaattgaacggtgaagctcgtgtggtgggcattgtggatcgcaattctgctattgaaatcgtcacacgtgaaaaggccaacccctctaaccccggtgacattggtgctcctatgtcgggtgtggttgtcgagatccgtgccaaggaaggtagccatgtcaaggccggtgatcctcttgctgttctctctgctatgaagatggaaacagtggtcactgctcccgtggctggtagagttgagcgtgttgctatccaagaaggtgattcattatccgctggtgatttggtggccaaggttgtcaaagaggaagcctaa

SEQ ID NO: 104 - DNA, 29 bp, Artificial
  trpCter-R
atgagaggcaaaatgaagcgtacaaagag

SEQ ID NO: 105 - DNA, 40 bp, Artificial
  trpCter-cicCpro-F
cattttgcctctcatcttacgcaggttgatagtagccgcc

SEQ ID NO: 106 - DNA, 40 bp, Artificial
  cipCpro-adhter-R
gcgtaattaaaatgaggttagagtatgaagaaaaaaaaaa

SEQ ID NO: 107 - DNA, 31 bp, Artificial
  trpC-lost-F2
tttaaatcttacgcaggttgatagtagccgc

SEQ ID NO: 108 - DNA, 33 bp, Artificial
  trpC-lost-R2
tgcgtaagatttaaatgaattcgagctcggtac

SEQ ID NO: 109 - DNA, 29 bp, Artificial
  cipCpro-R
ggttagagtatgaagaaaaaaaaaaaacg

SEQ ID NO: 110 - DNA, 45 bp, Artificial
  cipCpro-LifeTALEN-F
cttcatactctaaccatgggaaaacctattcctaatcctctgctg

SEQ ID NO: 111 - DNA, 40 bp, Artificial
  cipCpro-exo1-F
cttcatactctaaccatgaaaatccaagttgcttctccta

SEQ ID NO: 112 - DNA, 40 bp, Artificial
  pdc3-upstr-F
cggccagtgccaagcccgtcaggggtgaatgagatatttt

SEQ ID NO: 113 - DNA, 33 bp, Artificial
  pdc3-upstr-R2
aaaagatgtgagttataaaaggatgatgcaagc

SEQ ID NO: 114 - DNA, 33 bp, Artificial
  pdc3-downstr-F2
taactcacatcttttattctttttctatccctc

SEQ ID NO: 115 - DNA, 40 bp, Artificial
  pdc3-downstr-R
agagtcgacctgcagacctgttagaaaggtacatgcattc

SEQ ID NO: 116 - DNA, 40 bp, Artificial
  pdc3-upstr-R
cattttgcctctcatgtgagttataaaaggatgatgcaag

SEQ ID NO: 117 - DNA, 40 bp, Artificial
  pdc3-downstr-F
attaacttgctgttcatcttttattctttttctatccctc

SEQ ID NO: 118 - DNA, 23 bp, Artificial
  pdc3-upstr-F2
ccgtcaggggtgaatgagatatt

SEQ ID NO: 119 - DNA, 25 bp, Artificial
  pdc3-downstr-R2-P
acctgttagaaaggtacatgcattc

SEQ ID NO: 120 - DNA, 21 bp, Artificial
  pdc3-up
gacctcaatcactatccttgg

SEQ ID NO: 121 - DNA, 44 bp, Artificial
  pUC18-adh1pro-F
cggccagtgccaagcattattattagagggaaaaaaaagaaaga

SEQ ID NO: 122 - DNA, 44 bp, Artificial
  adh1pro-pUC18-R
agagtcgacctgcagttttgttatttatttgtattaattgataa

SEQ ID NO: 123 - DNA, 40 bp, Artificial
  adh1pro-adh1ter-F
aacaaaatcattttaattacgcattttcattttttactaa

SEQ ID NO: 124 - DNA, 44 bp, Artificial
  adh1ter-pUC18-R
agagtcgacctgcagagcagaacatgagtctggaagcgagacac

SEQ ID NO: 125 - DNA, 40 bp, Artificial
  adh1pro-adh1ter-R
taaaatgattttgttatttatttgtattaattgataatga

SEQ ID NO: 126 - DNA, 31 bp, Artificial
  adh1pro(o)-R
ttttgttatttatttgtattaattgataatg

SEQ ID NO: 127 - DNA, 30 bp, Artificial
  adh1ter(o)-F
tcattttaattacgcattttcattttttac

SEQ ID NO: 128 - DNA, 44 bp, Artificial
  adh1pro(o)-LifeTALEN-F
aaataaataacaaaaatgggaaaacctattcctaatcctctgct

SEQ ID NO: 129 - DNA, 44 bp, Artificial
  LifeTALEN-adh1ter(o)-R
gcgtaattaaaatgatcagaagttgatctcgccgttgttgaact

SEQ ID NO: 130 - DNA, 40 bp, Artificial
  ldhA-upstr-F
cggccagtgccaagcaaaagaataagaaaagatgtgtcag

SEQ ID NO: 131 - DNA, 32 bp, Artificial
  ldhA-upstr-R2
taaattaaggacttgagcttgaacgatgtcag

SEQ ID NO: 132 - DNA, 33 bp, Artificial
  ldhA-downstr-F2
caagtccttaatttacaaataataaatcatgtt

SEQ ID NO: 133 - DNA, 40 bp, Artificial
  ldhA-downstr-R
agagtcgacctgcagaacgacaaacatggctatcaaggga

SEQ ID NO: 134 - DNA, 40 bp, Artificial
  ldhA-upstr-R
tgtgcaagtgaacaaaggacttgagcttgaacgatgtcag

SEQ ID NO: 135 - DNA, 40 bp, Artificial
  ldhA-downstr-F
gctcttgacaatgcataatttacaaataataaatcatgtt

SEQ ID NO: 136 - DNA, 25 bp, Artificial
  ade1pro-R
tgcattgtcaagagcgtgtcgcaac

SEQ ID NO: 137 - DNA, 29 bp, Artificial
  ade1ter-F
ttgttcacttgcacagcgtgatatgcaag

SEQ ID NO: 138 - DNA, 28 bp, Artificial
  ldhA-upstr-F2
aaaagaataagaaaagatgtgtcaggac

SEQ ID NO: 139 - DNA, 27 bp, Artificial
  ldhA-downstr-R2-P
aacgacaaacatggctatcaagggaac

SEQ ID NO: 140 - DNA, 22 bp, Artificial
  ldhA-up
gaaactacagtattccctcgtg

SEQ ID NO: 141 - DNA, 21 bp, Artificial
  ade1-15
tgcttccatatgtcaataggc

SEQ ID NO: 142 - DNA, 40 bp, Artificial
  exo1-adhter-R2
gcgtaattaaaatgattatcttctttcatgagaaacacta

SEQ ID NO: 143 - DNA, 1749 bp, Rhizopus delemar
  pdc3
atggttagtatcaaaattggagattatctcattcaacgtcttaaagaaaccggaatcgacacgatttttggtgttccaggtgattacaatatggtaagttacgaagtggatacagatttatttgaatgtgtgtatatcctgaaaaactttgcaatgtagccgctattggatttaattgaagatgattctgagctcatatggggtaataatgcaaacgaactcaatgcttcctatgctgctgatggctatgctcgtatcagaggctttggtgctgtagttaccacgtttggtgtaggggaactttctgctgcagcaggtattgctggatcttattctgaaaaagtcccagtacttcatattgtcggcactcctaatactaaatcccaggaagctggagctattcttcatcacacgcttggtaatggcaattttcaggtgtttgttgaaatgttttccatgatcacgtgtgcttctactcatttaaactttgacaatgccatccgagaaattgatcgcgtcatccagcagactatgattcgaaagcgacctggttatatcggcatccccattgatctgattaatgctgaggttgctcttcctagttctgaacctctcaatttttttgtccccaaaaatcctactcaaactcaagatgtggctcttaaggttgttttggacgctatttcacaggctaagcatccgattatagttgttgatgcatgtgttcagcgacacaatttagttcaagaggctattgaattcgtgaaacgtaccggttttcccacttacgttgcacctatgggtaaaggtattgttcccgaggatcttgtcaattatcgtggttgctatgctggtaatattaccatcgagggtatcgccagggaacttgagcaagctgatctggtcattgaacttggtgcgattaaatccgatttcaacactggtggcttcacctataaactggatcctgctagaacgatctctcttcactcatttggtacccagatattttatgccgactatgacaaagtgggaatgacggaatttcttcctcttttgaccaagtctcttcctcaaaggcctcgtgtatttgatctaggccctcgtcatgagccagatccaattcaatcaggaactgaaataacgcacaattatttctggaataaggtaccagaatacatggatcctcgcgctgttgttgttgctgaaacaggcacagctgaatttgcctcttttaatttaagagctcccaaagacgctctctttatttctcaagtactctggggatccatcggttttgctgtcggatgtgctgtcggtgctgcgttcgctgatcgagatcgacgagtttatctttttgtgggtgatggctctttccaggttacttgtcaagaaatttcagtctttttgcatcaagggttgacacctgtcattttcttgttgaacaatgatggataccttatcgaaaaactcattcatgggcctcaccgctcttataataactttcagatgtggaactacagcaaaactcttgactatatgggtggacatcttcagcgcaatctgtctgatgtttcgccagctcaagttggtgttgaagctcaagtccgtacgcgagatgagtttgagagggcaatgaagacagtcaaggaggaacgtaacaaaattcattttattgaagttgtcatgcctcaatttgatgctcctcgcgaattgatactccaagttcaaacttctgaaaatcgttaa

SEQ ID NO: 144 - DNA, 3075 bp, Artificial Sequence
  LeftTALEN-pdc3
atgggaaaacctattcctaatcctctgctgggcctggattctaccggaggcatggcccctaagaaaaagcggaaggtggacggcggagtggacctgagaacactgggatattctcagcagcagcaggagaagatcaagcccaaggtgagatctacagtggcccagcaccacgaagccctggtgggacacggatttacacacgcccacattgtggccctgtctcagcaccctgccgccctgggaacagtggccgtgaaatatcaggatatgattgccgccctgcctgaggccacacacgaagccattgtgggagtgggaaaacgaggcgctggagccagagccctggaagccctgctgacagtggccggagaactgagaggacctcctctgcagctggatacaggacagctgctgaagattgccaaaaggggcggagtgaccgcggtggaagccgtgcacgcctggagaaatgccctgacaggagcccctctgaacctgacccccgaacaggtggtggccattgccagccacgacggcggcaagcaggccctggaaaccgtgcagagactgctgcccgtgctgtgccaggcccatggcctgacacctgaacaggtggtggctatcgcctctaacaacggaggaaaacaggctctggaaacagtgcagcggctgctgcctgtgctgtgtcaggctcacggcttgactccagaacaggtggtggctattgcttccaacaacggggggaaacaggccctggaaactgtgcagcgcctgctgccagtgctgtgccaggctcacggactgacccccgaacaggtggtggccattgccagcaacatcggcggcaagcaggccctggaaaccgtgcagagactgctgcccgtgctgtgccaggcccatggcctgacacctgaacaggtggtggctatcgcctctaatatcggaggaaaacaggctctggaaacagtgcagcggctgctgcctgtgctgtgtcaggctcacggcttgactccagaacaggtggtggctattgcttccaacggcggggggaaacaggccctggaaactgtgcagcgcctgctgccagtgctgtgccaggctcacgggctgacccccgaacaggtggtggccattgccagccacgacggcggcaagcaggccctggaaaccgtgcagagactgctgcccgtgctgtgccaggcccatggcctgacacctgaacaggtggtggctatcgcctctaacaacggaggaaaacaggctctggaaacagtgcagcggctgctgcctgtgctgtgtcaggctcacggcttgactccagaacaggtggtggctattgcttccaatattggggggaaacaggccctggaaactgtgcagcgcctgctgccagtgctgtgccaggctcacggcctcactcccgaacaggtggtggccattgccagccacgacggcggcaagcaggccctggaaaccgtgcagagactgctgcccgtgctgtgccaggcccatggcctgacacctgaacaggtggtggctatcgcctctaatatcggaggaaaacaggctctggaaacagtgcagcggctgctgcctgtgctgtgtcaggctcacggcttgactccagaacaggtggtggctattgcttcccacgacggggggaaacaggccctggaaactgtgcagcgcctgctgccagtgctgtgccaggctcacggactgacccccgaacaggtggtggccattgccagcaacaacggcggcaagcaggccctggaaaccgtgcagagactgctgcccgtgctgtgccaggcccatggcctgacacctgaacaggtggtggctatcgcctctaatatcggaggaaaacaagcactcgagacagtgcagcggctgctgcctgtgctgtgtcaggctcacggcttgactccagaacaggtggtggctattgcttccaacggcggggggaaacaggccctggaaactgtgcagcgcctgctgccagtgctgtgccaggctcacgggctgacccccgaacaggtggtggccattgccagcaacggcggcggcaagcaggccctggaaaccgtgcagagactgctgcccgtgctgtgccaggcccatggcctgacacctgaacaggtggtggctatcgcctctaacggcggaggaaaacaggctctggaaacagtgcagcggctgctgcctgtgctgtgtcaggctcacggcttgactccacagcaggtcgtggcaattgctagcaacggcggcggacggcccgccctggagagcattgtggcccagctgtctagacctgatcctgccctggccgccctgacaaatgatcacctggtggccctggcctgtctgggaggcagacctgccctggatgccgtgaaaaaaggactgcctcacgcccctgccctgatcaagagaacaaatagaagaatccccgagcggacctctcacagagtggccggatcccagctggtgaaatctgagctggaggagaagaagtctgagctgagacacaagctgaagtacgtgcctcacgagtacatcgagctgatcgagatcgccagaaatagcacccaggatagaatcctggagatgaaggtgatggagttcttcatgaaggtgtacggctacagaggaaagcacctgggaggaagcagaaaacctgacggagccatttatacagtgggcagccctatcgattatggcgtgatcgtggatacaaaggcctacagcggaggctacaatctgcctattggacaggccgatgagatgcagagatacgtggaggagaaccagaccaggaacaagcacatcaaccctaacgagtggtggaaggtgtacccttctagcgtgaccgagttcaagttcctgtttgtgagcggccacttcaagggcaattataaggcccagctgaccaggctgaaccacatcacaaattgtaatggcgccgtgctgtctgtggaggaactgctgattggaggagagatgattaaggccggaacactgacactggaggaggtgagaagaaagttcaacaacggcgagatcaacttctga

SEQ ID NO: 145 - DNA, 3075 bp, Artificial Sequence
  RightTALEN-pdc3
atgggaaaacctattcctaatcctctgctgggcctggattctaccggaggcatggcccctaagaaaaagcggaaggtggacggcggagtggacctgagaacactgggatattctcagcagcagcaggagaagatcaagcccaaggtgagatctacagtggcccagcaccacgaagccctggtgggacacggatttacacacgcccacattgtggccctgtctcagcaccctgccgccctgggaacagtggccgtgaaatatcaggatatgattgccgccctgcctgaggccacacacgaagccattgtgggagtgggaaaacgaggcgctggagccagagccctggaagccctgctgacagtggccggagaactgagaggacctcctctgcagctggatacaggacagctgctgaagattgccaaaaggggcggagtgaccgcggtggaagccgtgcacgcctggagaaatgccctgacaggagcccctctgaacctgacccccgaacaggtggtggccattgccagcaacaacggcggcaagcaggccctggaaaccgtgcagagactgctgcccgtgctgtgccaggcccatggcctgacacctgaacaggtggtggctatcgcctctaacggcggaggaaaacaggctctggaaacagtgcagcggctgctgcctgtgctgtgtcaggctcacggcttgactccagaacaggtggtggctattgcttccaatattggggggaaacaggccctggaaactgtgcagcgcctgctgccagtgctgtgccaggctcacggactgacccccgaacaggtggtggccattgccagcaacatcggcggcaagcaggccctggaaaccgtgcagagactgctgcccgtgctgtgccaggcccatggcctgacacctgaacaggtggtggctatcgcctctcacgacggaggaaaacaggctctggaaacagtgcagcggctgctgcctgtgctgtgtcaggctcacggcttgactccagaacaggtggtggctattgcttccaacggcggggggaaacaggccctggaaactgtgcagcgcctgctgccagtgctgtgccaggctcacgggctgacccccgaacaggtggtggccattgccagcaacggcggcggcaagcaggccctggaaaccgtgcagagactgctgcccgtgctgtgccaggcccatggcctgacacctgaacaggtggtggctatcgcctctaatatcggaggaaaacaggctctggaaacagtgcagcggctgctgcctgtgctgtgtcaggctcacggcttgactccagaacaggtggtggctattgcttcccacgacggggggaaacaggccctggaaactgtgcagcgcctgctgccagtgctgtgccaggctcacggcctcactcccgaacaggtggtggccattgccagccacgacggcggcaagcaggccctggaaaccgtgcagagactgctgcccgtgctgtgccaggcccatggcctgacacctgaacaggtggtggctatcgcctctaatatcggaggaaaacaggctctggaaacagtgcagcggctgctgcctgtgctgtgtcaggctcacggcttgactccagaacaggtggtggctattgcttccaacggcggggggaaacaggccctggaaactgtgcagcgcctgctgccagtgctgtgccaggctcacggactgacccccgaacaggtggtggccattgccagcaacatcggcggcaagcaggccctggaaaccgtgcagagactgctgcccgtgctgtgccaggcccatggcctgacacctgaacaggtggtggctatcgcctctaacggcggaggaaaacaagcactcgagacagtgcagcggctgctgcctgtgctgtgtcaggctcacggcttgactccagaacaggtggtggctattgcttccaacggcggggggaaacaggccctggaaactgtgcagcgcctgctgccagtgctgtgccaggctcacgggctgacccccgaacaggtggtggccattgccagcaacaacggcggcaagcaggccctggaaaccgtgcagagactgctgcccgtgctgtgccaggcccatggcctgacacctgaacaggtggtggctatcgcctctaacggcggaggaaaacaggctctggaaacagtgcagcggctgctgcctgtgctgtgtcaggctcacggcttgactccacagcaggtcgtggcaattgctagcaatatcggcggacggcccgccctggagagcattgtggcccagctgtctagacctgatcctgccctggccgccctgacaaatgatcacctggtggccctggcctgtctgggaggcagacctgccctggatgccgtgaaaaaaggactgcctcacgcccctgccctgatcaagagaacaaatagaagaatccccgagcggacctctcacagagtggccggatcccagctggtgaaatctgagctggaggagaagaagtctgagctgagacacaagctgaagtacgtgcctcacgagtacatcgagctgatcgagatcgccagaaatagcacccaggatagaatcctggagatgaaggtgatggagttcttcatgaaggtgtacggctacagaggaaagcacctgggaggaagcagaaaacctgacggagccatttatacagtgggcagccctatcgattatggcgtgatcgtggatacaaaggcctacagcggaggctacaatctgcctattggacaggccgatgagatgcagagatacgtggaggagaaccagaccaggaacaagcacatcaaccctaacgagtggtggaaggtgtacccttctagcgtgaccgagttcaagttcctgtttgtgagcggccacttcaagggcaattataaggcccagctgaccaggctgaaccacatcacaaattgtaatggcgccgtgctgtctgtggaggaactgctgattggaggagagatgattaaggccggaacactgacactggaggaggtgagaagaaagttcaacaacggcgagatcaacttctga

SEQ ID NO: 146 - DNA, 19 bp, Rhizopus delemar
  Target of LeftTALEN-pdc3
ccggaatcgacacgatttt

SEQ ID NO: 147 - DNA, 19 bp, Rhizopus delemar
  Target of RightTALEN-pdc3
cgtaacttaccatattgta

SEQ ID NO: 148 - DNA, 963 bp, Rhizopus oryzae
  ldhA
atggtattacactcaaaggtcgccatcgttggagctggtgcagtaggagcctccactgcttatgcacttatgtttaaaaacatttgtacagaaatcattattgttgatgttaatcctgacatcgttcaagctcaagtccttgaccttgcagatgctgccagtataagtcacacgcccatccgagcaggtagcgcagaggaggcagggcaggcagatattgttgtcatcacggccggtgcgaaacaaagggaaggtgagcctcggacaaagctcattgaacgaaacttcagagtgttgcaaagtatcattggtggcatgcaacccattcgaccagacgcagtcatcttggtggtagcaaatccagtcgatatcttgacacacattgcaaagaccctctctggactgcctccaaaccaggtcattggctccggtacctaccttgacacgacccgtcttcgcgtccatcttggcgatgtctttgatgtcaatcctcaatcggtccatgcttttgtcttgggtgaacatggggattcccagatgatcgcttgggaggctgcttcgattggtggccagccgttgacaagtttcccggaattcgcaaagctggataaaacagcaatttcaaaagcgatatcaggtaaagcgatggagatcattcgtttgaaaggagccacgttttatggaattggtgcctgtgcagcggatttagtgcacactatcatgttgaataggaaatcagtacatccagtttctgtttatgttgaaaagtatggagccactttttctatgcctgctaaacttggatggagaggtgttgaacagatctatgaagtaccactgacggaagaagaagaagcgttgcttgtaaaatctgtagaggcattgaaatcagttgaatattcatctacaaaagttccagaaaaaaaggttcatgctacttccttttctaaaagtagctgttga

SEQ ID NO: 149 - DNA, 3075 bp, Artificial Sequence
  LeftTALEN-ldhA
atgggaaaacctattcctaatcctctgctgggcctggattctaccggaggcatggcccctaagaaaaagcggaaggtggacggcggagtggacctgagaacactgggatattctcagcagcagcaggagaagatcaagcccaaggtgagatctacagtggcccagcaccacgaagccctggtgggacacggatttacacacgcccacattgtggccctgtctcagcaccctgccgccctgggaacagtggccgtgaaatatcaggatatgattgccgccctgcctgaggccacacacgaagccattgtgggagtgggaaaacagtggtctggagccagagccctggaagccctgctgacagtggccggagaactgagaggacctcctctgcagctggatacaggacagctgctgaagattgccaaaaggggcggagtgaccgcggtggaagccgtgcacgcctggagaaatgccctgacaggagcccctctgaacctgacccccgaacaggtggtggccattgccagcaacaacggcggcaagcaggccctggaaaccgtgcagagactgctgcccgtgctgtgccaggcccatggcctgacacctgaacaggtggtggctatcgcctctcacgacggaggaaaacaggctctggaaacagtgcagcggctgctgcctgtgctgtgtcaggctcacggcttgactccagaacaggtggtggctattgcttccaatattggggggaaacaggccctggaaactgtgcagcgcctgctgccagtgctgtgccaggctcacggactgacccccgaacaggtggtggccattgccagcaacaacggcggcaagcaggccctggaaaccgtgcagagactgctgcccgtgctgtgccaggcccatggcctgacacctgaacaggtggtggctatcgcctctaatatcggaggaaaacaggctctggaaacagtgcagcggctgctgcctgtgctgtgtcaggctcacggcttgactccagaacaggtggtggctattgcttccaacggcggggggaaacaggccctggaaactgtgcagcgcctgctgccagtgctgtgccaggctcacgggctgacccccgaacaggtggtggccattgccagcaacaacggcggcaagcaggccctggaaaccgtgcagagactgctgcccgtgctgtgccaggcccatggcctgacacctgaacaggtggtggctatcgcctctcacgacggaggaaaacaggctctggaaacagtgcagcggctgctgcctgtgctgtgtcaggctcacggcttgactccagaacaggtggtggctattgcttccaacggcggggggaaacaggccctggaaactgtgcagcgcctgctgccagtgctgtgccaggctcacggcctcactcccgaacaggtggtggccattgccagcaacaacggcggcaagcaggccctggaaaccgtgcagagactgctgcccgtgctgtgccaggcccatggcctgacacctgaacaggtggtggctatcgcctctcacgacggaggaaaacaggctctggaaacagtgcagcggctgctgcctgtgctgtgtcaggctcacggcttgactccagaacaggtggtggctattgcttcccacgacggggggaaacaggccctggaaactgtgcagcgcctgctgccagtgctgtgccaggctcacggactgacccccgaacaggtggtggccattgccagcaacatcggcggcaagcaggccctggaaaccgtgcagagactgctgcccgtgctgtgccaggcccatggcctgacacctgaacaggtggtggctatcgcctctaacaacggaggaaaacaagcactcgagacagtgcagcggctgctgcctgtgctgtgtcaggctcacggcttgactccagaacaggtggtggctattgcttccaacggcggggggaaacaggccctggaaactgtgcagcgcctgctgccagtgctgtgccaggctcacgggctgacccccgaacaggtggtggccattgccagcaacatcggcggcaagcaggccctggaaaccgtgcagagactgctgcccgtgctgtgccaggcccatggcctgacacctgaacaggtggtggctatcgcctctaacggcggaggaaaacaggctctggaaacagtgcagcggctgctgcctgtgctgtgtcaggctcacggcttgactccacagcaggtcgtggcaattgctagcaatatcggcggacggcccgccctggagagcattgtggcccagctgtctagacctgatcctgccctggccgccctgacaaatgatcacctggtggccctggcctgtctgggaggcagacctgccctggatgccgtgaaaaaaggactgcctcacgcccctgccctgatcaagagaacaaatagaagaatccccgagcggacctctcacagagtggccggatcccagctggtgaaatctgagctggaggagaagaagtctgagctgagacacaagctgaagtacgtgcctcacgagtacatcgagctgatcgagatcgccagaaatagcacccaggatagaatcctggagatgaaggtgatggagttcttcatgaaggtgtacggctacagaggaaagcacctgggaggaagcagaaaacctgacggagccatttatacagtgggcagccctatcgattatggcgtgatcgtggatacaaaggcctacagcggaggctacaatctgcctattggacaggccgatgagatgcagagatacgtggaggagaaccagaccaggaacaagcacatcaaccctaacgagtggtggaaggtgtacccttctagcgtgaccgagttcaagttcctgtttgtgagcggccacttcaagggcaattataaggcccagctgaccaggctgaaccacatcacaaattgtaatggcgccgtgctgtctgtggaggaactgctgattggaggagagatgattaaggccggaacactgacactggaggaggtgagaagaaagttcaacaacggcgagatcaacttctga

SEQ ID NO: 150 - DNA, 3075 bp, Artificial Sequence
  RightTALEN-ldhA
atgggaaaacctattcctaatcctctgctgggcctggattctaccggaggcatggcccctaagaaaaagcggaaggtggacggcggagtggacctgagaacactgggatattctcagcagcagcaggagaagatcaagcccaaggtgagatctacagtggcccagcaccacgaagccctggtgggacacggatttacacacgcccacattgtggccctgtctcagcaccctgccgccctgggaacagtggccgtgaaatatcaggatatgattgccgccctgcctgaggccacacacgaagccattgtgggagtgggaaaacagtggtctggagccagagccctggaagccctgctgacagtggccggagaactgagaggacctcctctgcagctggatacaggacagctgctgaagattgccaaaaggggcggagtgaccgcggtggaagccgtgcacgcctggagaaatgccctgacaggagcccctctgaacctgacccccgaacaggtggtggccattgccagccacgacggcggcaagcaggccctggaaaccgtgcagagactgctgcccgtgctgtgccaggcccatggcctgacacctgaacaggtggtggctatcgcctctcacgacggaggaaaacaggctctggaaacagtgcagcggctgctgcctgtgctgtgtcaggctcacggcttgactccagaacaggtggtggctattgcttccaacggcggggggaaacaggccctggaaactgtgcagcgcctgctgccagtgctgtgccaggctcacggactgacccccgaacaggtggtggccattgccagccacgacggcggcaagcaggccctggaaaccgtgcagagactgctgcccgtgctgtgccaggcccatggcctgacacctgaacaggtggtggctatcgcctctaacggcggaggaaaacaggctctggaaacagtgcagcggctgctgcctgtgctgtgtcaggctcacggcttgactccagaacaggtggtggctattgcttccaacaacggggggaaacaggccctggaaactgtgcagcgcctgctgccagtgctgtgccaggctcacgggctgacccccgaacaggtggtggccattgccagccacgacggcggcaagcaggccctggaaaccgtgcagagactgctgcccgtgctgtgccaggcccatggcctgacacctgaacaggtggtggctatcgcctctaacaacggaggaaaacaggctctggaaacagtgcagcggctgctgcctgtgctgtgtcaggctcacggcttgactccagaacaggtggtggctattgcttcccacgacggggggaaacaggccctggaaactgtgcagcgcctgctgccagtgctgtgccaggctcacggcctcactcccgaacaggtggtggccattgccagcaacggcggcggcaagcaggccctggaaaccgtgcagagactgctgcccgtgctgtgccaggcccatggcctgacacctgaacaggtggtggctatcgcctctaatatcggaggaaaacaggctctggaaacagtgcagcggctgctgcctgtgctgtgtcaggctcacggcttgactccagaacaggtggtggctattgcttcccacgacggggggaaacaggccctggaaactgtgcagcgcctgctgccagtgctgtgccaggctcacggactgacccccgaacaggtggtggccattgccagccacgacggcggcaagcaggccctggaaaccgtgcagagactgctgcccgtgctgtgccaggcccatggcctgacacctgaacaggtggtggctatcgcctctaacggcggaggaaaacaagcactcgagacagtgcagcggctgctgcctgtgctgtgtcaggctcacggcttgactccagaacaggtggtggctattgcttccaacaacggggggaaacaggccctggaaactgtgcagcgcctgctgccagtgctgtgccaggctcacgggctgacccccgaacaggtggtggccattgccagccacgacggcggcaagcaggccctggaaaccgtgcagagactgctgcccgtgctgtgccaggcccatggcctgacacctgaacaggtggtggctatcgcctctaacggcggaggaaaacaggctctggaaacagtgcagcggctgctgcctgtgctgtgtcaggctcacggcttgactccacagcaggtcgtggcaattgctagccacgacggcggacggcccgccctggagagcattgtggcccagctgtctagacctgatcctgccctggccgccctgacaaatgatcacctggtggccctggcctgtctgggaggcagacctgccctggatgccgtgaaaaaaggactgcctcacgcccctgccctgatcaagagaacaaatagaagaatccccgagcggacctctcacagagtggccggatcccagctggtgaaatctgagctggaggagaagaagtctgagctgagacacaagctgaagtacgtgcctcacgagtacatcgagctgatcgagatcgccagaaatagcacccaggatagaatcctggagatgaaggtgatggagttcttcatgaaggtgtacggctacagaggaaagcacctgggaggaagcagaaaacctgacggagccatttatacagtgggcagccctatcgattatggcgtgatcgtggatacaaaggcctacagcggaggctacaatctgcctattggacaggccgatgagatgcagagatacgtggaggagaaccagaccaggaacaagcacatcaaccctaacgagtggtggaaggtgtacccttctagcgtgaccgagttcaagttcctgtttgtgagcggccacttcaagggcaattataaggcccagctgaccaggctgaaccacatcacaaattgtaatggcgccgtgctgtctgtggaggaactgctgattggaggagagatgattaaggccggaacactgacactggaggaggtgagaagaaagttcaacaacggcgagatcaacttctga

SEQ ID NO: 151 - DNA, 19 bp, Rhizopus oryzae
  Target of LeftTALEN-ldhA
tgcagatgctgccagtata

SEQ ID NO: 152 - DNA, 19 bp, Rhizopus oryzae
  Target of RightTALEN-ldhA
tcctctgcgctacctgctc